European Patent Application EP 4 741 401 A1, published May 13, 2026. Title: Benzothiazoimidazolyl compound and use thereof. Applicant: 小胞体ストレス研究所株式会社. The sequence listing filed with the application follows.

SEQUENCE LISTING (3 sequences)

SEQ ID NO: 1 - DNA, 32 bp, human
  source 1..32: mol_type = genomic DNA
ggcgccgattgggccacgttgggagagtgcct

SEQ ID NO: 2 - DNA, 27 bp, human
  source 1..27: mol_type = genomic DNA
ctcgagacaggtgctgacgtggcattc

SEQ ID NO: 3 - DNA, 19 bp, human
  source 1..19: mol_type = genomic DNA
aacattgcatcatccccgc